European Patent Specification EP 3 765 519 B1, published January 17, 2024. Title: ANTI-CXCR4 ANTIBODY COMBINED WITH ACTIVATED AND EXPANDED NATURAL KILLER CELLS FOR CANCER IMMUNOTHERAPY. Applicant: FUNDACIÓN PARA LA LNVESTIGACIÓN BIOMÉDICA DEL HOSPITAL UNIVERSITARIO LA PAZ (FIBHULP). The sequence listing filed with the application follows.

SEQUENCE LISTING (43 sequences)

SEQ ID NO: 1 - protein, 5 aa, Homo sapiens
SYSMN

SEQ ID NO: 2 - protein, 5 aa, Homo sapiens
SYSMN

SEQ ID NO: 3 - protein, 5 aa, Homo sapiens
SYSMN

SEQ ID NO: 4 - protein, 5 aa, Homo sapiens
SYSMN

SEQ ID NO: 5 - protein, 17 aa, Homo sapiens
YISSRSRTIYYADSVKG

SEQ ID NO: 6 - protein, 17 aa, Homo sapiens
YISSRSRSIYYADSVKG

SEQ ID NO: 7 - protein, 17 aa, Homo sapiens
YISSRSKTIYYADSVKG

SEQ ID NO: 8 - protein, 17 aa, Homo sapiens
YISSRSRTIYYADSVKG

SEQ ID NO: 9 - protein, 16 aa, Homo sapiens
DYGGQPPYYYYYGMDV

SEQ ID NO: 10 - protein, 16 aa, Homo sapiens
DYGGQPPYYYYYGMDV

SEQ ID NO: 11 - protein, 16 aa, Homo sapiens
DYGGQPPYYYYYGMDV

SEQ ID NO: 12 - protein, 16 aa, Homo sapiens
DYGGQPPYHYYYGMDV

SEQ ID NO: 13 - protein, 11 aa, Homo sapiens
RASQGISSWLA

SEQ ID NO: 14 - protein, 11 aa, Homo sapiens
RASQGISSWLA

SEQ ID NO: 15 - protein, 11 aa, Homo sapiens
RTSQGISSWLA

SEQ ID NO: 16 - protein, 11 aa, Homo sapiens
RASQGISNWLA

SEQ ID NO: 17 - protein, 7 aa, Homo sapiens
AASSLQS

SEQ ID NO: 18 - protein, 7 aa, Homo sapiens
AASSLQS

SEQ ID NO: 19 - protein, 7 aa, Homo sapiens
AASSLQS

SEQ ID NO: 20 - protein, 7 aa, Homo sapiens
AASSLQS

SEQ ID NO: 21 - protein, 9 aa, Homo sapiens
QQYNSYPRT

SEQ ID NO: 22 - protein, 9 aa, Homo sapiens
QQYNSYPRT

SEQ ID NO: 23 - protein, 9 aa, Homo sapiens
QQYNSYPRT

SEQ ID NO: 24 - protein, 9 aa, Homo sapiens
QQYNSYPRT

SEQ ID NO: 25 - protein, 125 aa, Homo sapiens
QVQLVQSGGGLVQPGGSLRLSCAAAGFTFSSYSMNWVRQAPGKGLEWVSYISSRSRTIYYADSVKGRFTISRDNAKNSLYLQMNSLRDEDTAVYYCARDYGGQPPYYYYYGMDVWGQGTTVTVSS

SEQ ID NO: 26 - protein, 125 aa, Homo sapiens
QVQLVQSGGGLVQPGGSLRLSCAAAGFTFSSYSMNWVRQAPGKGLEWVSYISSRSRSIYYADSVKGRFTISRDNAKNSLYLQMNSLRDEDTAVYYCARDYGGQPPYYYYYGMDVWGQGTTVTVSS

SEQ ID NO: 27 - protein, 125 aa, Homo sapiens
EVQLVQSGGGLVQPGGSLRLSCAAAGFTFSSYSMNWVRQAPGKGLEWVSYISSRSKTIYYADSVKGRFTISRDNARNSLYLQMNSLRDEDTAVYYCARDYGGQPPYYYYYGMDVWGQGTTVTVSS

SEQ ID NO: 28 - protein, 125 aa, Homo sapiens
EVQLVQSGGGLVQPGGSLRLSCAAAGFTFSSYSMNWVRQAPGKGLEWVSYISSRSRTIYYADSVKGRFTISRDNAKNSLYLQMNSLRDEDTAVYYCARDYGGQPPYHYYYGMDVWGQGTTVTVSS

SEQ ID NO: 29 - protein, 107 aa, Homo sapiens
AIRMTQSPSSLSASVGDRVTITCRASQGISSWLAWYQQKPEKAPKSLIYAASSLQSGVPSRFSGSGSGTDFTLTISSLQPEDFVTYYCQQYNSYPRTFGQGTKVEIK

SEQ ID NO: 30 - protein, 107 aa, Homo sapiens
EIVLTQSPSSLSASVGDRVTITCRASQGISSWLAWYQQKPEKAPKSLIYAASSLQSGVPPRFSGSGSGTDFTLTISSLQPEDFATYYCQQYNSYPRTFGQGTKVEIK

SEQ ID NO: 31 - protein, 107 aa, Homo sapiens
VIWVTQSPSSLSASVGDRVTITCRTSQGISSWLAWYQQKPEKAPELLIYAASSLQSGVPSRFSGSGSGTDFTLTISSLQPEDFATYYCQQYNSYPRTFGQGTKVEIK

SEQ ID NO: 32 - protein, 107 aa, Homo sapiens
EIVLTQSPSSLSASVGDRVTITCRASQGISNWLAWYQQKPEKAPKSLIYAASSLQSGVPSRFSGSGSGTDFTLTISSLQPEDFATYYCQQYNSYPRTFGQGTKVEIK

SEQ ID NO: 33 - protein, 125 aa, Homo sapiens
EVQLVESGGGLVQPGGSLRLSCAAAGFTFSSYSMNWVRQAPGKGLEWVSYISSRSRTIYYADSVKGRFTISRDNAKNSLYLQMNSLRDEDTAVYYCARDYGGQPPYYYYYGMDVWGQGTTVTVSS

SEQ ID NO: 34 - protein, 125 aa, Homo sapiens
EVQLVESGGGLVQPGGSLRLSCAAAGFTFSSYSMNWVRQAPGKGLEWVSYISSRSRSIYYADSVKGRFTISRDNAKNSLYLQMNSLRDEDTAVYYCARDYGGQPPYYYYYGMDVWGQGTTVTVSS

SEQ ID NO: 35 - protein, 125 aa, Homo sapiens
EVQLVESGGGLVQPGGSLRLSCAAAGFTFSSYSMNWVRQAPGKGLEWVSYISSRSKTIYYADSVKGRFTISRDNARNSLYLQMNSLRDEDTAVYYCARDYGGQPPYYYYYGMDVWGQGTTVTVSS

SEQ ID NO: 36 - protein, 125 aa, Homo sapiens; identical to SEQ ID NO: 28

SEQ ID NO: 37 - protein, 107 aa, Homo sapiens
DIQMTQSPSSLSASVGDRVTITCRASQGISSWLAWYQQKPEKAPKSLIYAASSLQSGVPSRFSGSGSGTDFTLTISSLQPEDFVTYYCQQYNSYPRTFGQGTKVEIK

SEQ ID NO: 38 - protein, 107 aa, Homo sapiens
DIQMTQSPSSLSASVGDRVTITCRASQGISSWLAWYQQKPEKAPKSLIYAASSLQSGVPPRFSGSGSGTDFTLTISSLQPEDFATYYCQQYNSYPRTFGQGTKVEIK

SEQ ID NO: 39 - protein, 107 aa, Homo sapiens
DIQMTQSPSSLSASVGDRVTITCRTSQGISSWLAWYQQKPEKAPELLIYAASSLQSGVPSRFSGSGSGTDFTLTISSLQPEDFATYYCQQYNSYPRTFGQGTKVEIK

SEQ ID NO: 40 - protein, 107 aa, Homo sapiens
DIQMTQSPSSLSASVGDRVTITCRASQGISNWLAWYQQKPEKAPKSLIYAASSLQSGVPSRFSGSGSGTDFTLTISSLQPEDFATYYCQQYNSYPRTFGQGTKVEIK

SEQ ID NO: 41 - protein, 98 aa, Homo sapiens
EVQLVESGGGLVQPGGSLRLSCAASGFTFSSYSMNWVRQAPGKGLEWVSYISSSSSTIYYADSVKGRFTISRDNAKNSLYLQMNSLRDEDTAVYYCAR

SEQ ID NO: 42 - protein, 95 aa, Homo sapiens
DIQMTQSPSSLSASVGDRVTITCRASQGISSWLAWYQQKPEKAPKSLIYAASSLQSGVPSRFSGSGSGTDFTLTISSLQPEDFATYYCQQYNSYP

SEQ ID NO: 43 - protein, 352 aa, Homo sapiens
MEGISIYTSDNYTEEMGSGDYDSMKEPCFREENANFNKIFLPTIYSIIFLTGIVGNGLVILVMGYQKKLRSMTDKYRLHLSVADLLFVITLPFWAVDAVANWYFGNFLCKAVHVIYTVNLYSSVLILAFISLDRYLAIVHATNSQRPRKLLAEKVVYVGVWIPALLLTIPDFIFANVSEADDRYICDRFYPNDLWVVVFQFQHIMVGLILPGIVILSCYCIIISKLSHSKGHQKRKALKTTVILILAFFACWLPYYIGISIDSFILLEIIKQGCEFENTVHKWISITEALAFFHCCLNPILYAFLGAKFKTSAQHALTSVSRGSSLKILSKGKRGGHSSVSTESESSSFHSS